European Patent Specification EP 3 823 657 B1, published June 5, 2024. Title: COMPOSITIONS A USAGE COSMETIQUE ET DERMATOLOGIQUE. Applicant: SEMIOCARE. The sequence listing filed with the application follows.

SEQUENCE LISTING (6 sequences)

SEQ ID NO: 1 - protein, 10 aa, Bos taurus
YLGYLEQLLR

SEQ ID NO: 2 - protein, 9 aa, Bos taurus
YLGYLEQLL

SEQ ID NO: 3 - protein, 8 aa, Bos taurus
YLGYLEQL

SEQ ID NO: 4 - protein, 7 aa, Bos taurus
YLGYLEQ

SEQ ID NO: 5 - protein, 6 aa, Bos taurus
YLGYLE

SEQ ID NO: 6 - protein, 5 aa, Bos taurus
YLGYL